European Patent Application EP 4 219 532 A2, published August 2, 2023. Title: COMPOSITIONS AND METHODS FOR TRANSIENT GENE THERAPY WITH ENHANCED STABILITY. Applicant: Dana-Farber Cancer Institute, Inc. The sequence listing filed with the application follows.

SEQUENCE LISTING (69 sequences)

SEQ ID NO: 1 - DNA, 20 bp, synthetic construct
  source 1..20: mol_type = other DNA
  misc_feature 1..20: note = Synthetic Polynucleotide
tggctgcacgaattgcacaa

SEQ ID NO: 2 - DNA, 20 bp, synthetic construct
  source 1..20: mol_type = other DNA
  misc_feature 1..20: note = Synthetic Polynucleotide
ttgtgcaattcgtgcagcca

SEQ ID NO: 3 - DNA, 20 bp, synthetic construct
  misc_feature 1..20: note = Synthetic Polynucleotide
  source 1..20: mol_type = other DNA
taatacgactcactataggg

SEQ ID NO: 4 - DNA, 10 bp, synthetic construct
  misc_feature 1..10: note = Synthetic Polynucleotide
  source 1..10: mol_type = other DNA
ttatgataac

SEQ ID NO: 5 - DNA, 10 bp, synthetic construct
  misc_feature 1..10: note = Synthetic Polynucleotide
  source 1..10: mol_type = other DNA
agcgacttcg

SEQ ID NO: 6 - DNA, 10 bp, synthetic construct
  misc_feature 1..10: note = Synthetic Polynucleotide
  source 1..10: mol_type = other DNA
aaaagaagga

SEQ ID NO: 7 - DNA, 10 bp, synthetic construct
  misc_feature 1..10: note = Synthetic Polynucleotide
  source 1..10: mol_type = other DNA
gagggaggga

SEQ ID NO: 8 - DNA, 40 bp, synthetic construct
  misc_feature 1..40: note = Synthetic Polynucleotide
  source 1..40: mol_type = other DNA
cgaagtcgcttggctgcacgaattgcacaatccctccctc

SEQ ID NO: 9 - DNA, 17 bp, synthetic construct
  misc_feature 1..17: note = Synthetic Polynucleotide
  source 1..17: mol_type = other DNA
taatacgactcactata

SEQ ID NO: 10 - DNA, 10 bp, synthetic construct
  misc_feature 1..10: note = Synthetic Polynucleotide
  source 1..10: mol_type = other DNA
cccccccccc

SEQ ID NO: 11 - DNA, 40 bp, synthetic construct
  misc_feature 1..40: note = Synthetic Polynucleotide
  source 1..40: mol_type = other DNA
cccccccccccccccccccccccccccccccccccccccc

SEQ ID NO: 12 - DNA, 10 bp, synthetic construct
  misc_feature 1..10: note = Synthetic Polynucleotide
  source 1..10: mol_type = other DNA
gggggggggg

SEQ ID NO: 13 - DNA, 40 bp, synthetic construct
  misc_feature 1..40: note = Synthetic Polynucleotide
  source 1..40: mol_type = other DNA
gggggggggggggggggggggggggggggggggggggggg

SEQ ID NO: 14 - DNA, 10 bp, synthetic construct
  misc_feature 1..10: note = Synthetic Polynucleotide
  source 1..10: mol_type = other DNA
aaaaaaaaaa

SEQ ID NO: 15 - DNA, 15 bp, synthetic construct
  misc_feature 1..15: note = Synthetic Polynucleotide
  source 1..15: mol_type = other DNA
aaaaaaaaaaaaaaa

SEQ ID NO: 16 - DNA, 20 bp, synthetic construct
  misc_feature 1..20: note = Synthetic Polynucleotide
  source 1..20: mol_type = other DNA
aaaaaaaaaaaaaaaaaaaa

SEQ ID NO: 17 - DNA, 10 bp, synthetic construct
  misc_feature 1..10: note = Synthetic Polynucleotide
  source 1..10: mol_type = other DNA
accgacggca

SEQ ID NO: 18 - DNA, 10 bp, synthetic construct
  misc_feature 1..10: note = Synthetic Polynucleotide
  source 1..10: mol_type = other DNA
tgccgtcggt

SEQ ID NO: 19 - DNA, 20 bp, synthetic construct
  misc_feature 1..20: note = Synthetic Polynucleotide
  source 1..20: mol_type = other DNA
aacacgttattgccgtcggt

SEQ ID NO: 20 - DNA, 20 bp, synthetic construct
  misc_feature 1..20: note = Synthetic Polynucleotide
  source 1..20: mol_type = other DNA
accgacggcaataacgtgtt

SEQ ID NO: 21 - DNA, 30 bp, synthetic construct
  misc_feature 1..30: note = Synthetic Polynucleotide
  source 1..30: mol_type = other DNA
accgacggcaataacgtgttggtacgtaac

SEQ ID NO: 22 - DNA, 40 bp, synthetic construct
  misc_feature 1..40: note = Synthetic Polynucleotide
  source 1..40: mol_type = other DNA
accgacggcaataacgtgttggtacgtaaccttcgaacct

SEQ ID NO: 23 - DNA, 40 bp, synthetic construct
  misc_feature 1..40: note = Synthetic Polynucleotide
  source 1..40: mol_type = other DNA
aggttcgaaggttacgtaccaacacgttattgccgtcggt

SEQ ID NO: 24 - DNA, 10 bp, synthetic construct
  misc_feature 1..10: note = Synthetic Polynucleotide
  source 1..10: mol_type = other DNA
cggaatatag

SEQ ID NO: 25 - DNA, 15 bp, synthetic construct
  misc_feature 1..15: note = Synthetic Polynucleotide
  source 1..15: mol_type = other DNA
cggaatatagaagca

SEQ ID NO: 26 - DNA, 20 bp, synthetic construct
  misc_feature 1..20: note = Synthetic Polynucleotide
  source 1..20: mol_type = other DNA
cggaatatagaagcataaga

SEQ ID NO: 27 - DNA, 10 bp, synthetic construct
  misc_feature 1..10: note = Synthetic Polynucleotide
  source 1..10: mol_type = other DNA
gggaaaaaaa

SEQ ID NO: 28 - DNA, 15 bp, synthetic construct
  misc_feature 1..15: note = Synthetic Polynucleotide
  source 1..15: mol_type = other DNA
gggaaaaaaaaaaaa

SEQ ID NO: 29 - DNA, 20 bp, synthetic construct
  misc_feature 1..20: note = Synthetic Polynucleotide
  source 1..20: mol_type = other DNA
gggaaaaaaaaaaaaaaaaa

SEQ ID NO: 30 - DNA, 10 bp, synthetic construct
  misc_feature 1..10: note = Synthetic Polynucleotide
  source 1..10: mol_type = other DNA
gggaatcgac

SEQ ID NO: 31 - DNA, 15 bp, synthetic construct
  misc_feature 1..15: note = Synthetic Polynucleotide
  source 1..15: mol_type = other DNA
gggaatcgactacag

SEQ ID NO: 32 - DNA, 20 bp, synthetic construct
  misc_feature 1..20: note = Synthetic Polynucleotide
  source 1..20: mol_type = other DNA
gggaatcgactacaggagga

SEQ ID NO: 33 - DNA, 30 bp, synthetic construct
  misc_feature 1..30: note = Synthetic Polynucleotide
  source 1..30: mol_type = other DNA
gttacgtaccaacacgttattgccgtcggt

SEQ ID NO: 34 - DNA, 40 bp, synthetic construct
  misc_feature 1..40: note = Synthetic Polynucleotide
  source 1..40: mol_type = other DNA
ctatattccgaacacgttattgccgtcggttccctccctc

SEQ ID NO: 35 - DNA, 60 bp, synthetic construct
  misc_feature 1..60: note = Synthetic Polynucleotide
  source 1..60: mol_type = other DNA
ctatattccgaggttcgaaggttacgtaccaacacgttattgccgtcggttccctccctc

SEQ ID NO: 36 - DNA, 30 bp, synthetic construct
  misc_feature 1..30: note = Synthetic Polynucleotide
  source 1..30: mol_type = other DNA
ctatattccgcccccccccctccctccctc

SEQ ID NO: 37 - DNA, 60 bp, synthetic construct
  misc_feature 1..60: note = Synthetic Polynucleotide
  source 1..60: mol_type = other DNA
ctatattccgcccccccccccccccccccccccccccccccccccccccctccctccctc

SEQ ID NO: 38 - DNA, 50 bp, synthetic construct
  misc_feature 1..50: note = Synthetic Polynucleotide
  source 1..50: mol_type = other DNA
ctatattccggttacgtaccaacacgttattgccgtcggttccctccctc

SEQ ID NO: 39 - DNA, 30 bp, synthetic construct
  misc_feature 1..30: note = Synthetic Polynucleotide
  source 1..30: mol_type = other DNA
ctatattccgtgccgtcggttccctccctc

SEQ ID NO: 40 - DNA, 50 bp, synthetic construct
  misc_feature 1..50: note = Synthetic Polynucleotide
  source 1..50: mol_type = other DNA
tcttatgcttctatattccgaacacgttattgccgtcggttccctccctc

SEQ ID NO: 41 - DNA, 70 bp, synthetic construct
  misc_feature 1..70: note = Synthetic Polynucleotide
  source 1..70: mol_type = other DNA
tcttatgcttctatattccgaggttcgaaggttacgtaccaacacgttattgccgtcggttccctccctc

SEQ ID NO: 42 - DNA, 70 bp, synthetic construct
  misc_feature 1..70: note = Synthetic Polynucleotide
  source 1..70: mol_type = other DNA
tcttatgcttctatattccgcccccccccccccccccccccccccccccccccccccccctccctccctc

SEQ ID NO: 43 - DNA, 40 bp, synthetic construct
  misc_feature 1..40: note = Synthetic Polynucleotide
  source 1..40: mol_type = other DNA
tcttatgcttctatattccgcccccccccctccctccctc

SEQ ID NO: 44 - DNA, 60 bp, synthetic construct
  misc_feature 1..60: note = Synthetic Polynucleotide
  source 1..60: mol_type = other DNA
tcttatgcttctatattccggttacgtaccaacacgttattgccgtcggttccctccctc

SEQ ID NO: 45 - DNA, 40 bp, synthetic construct
  misc_feature 1..40: note = Synthetic Polynucleotide
  source 1..40: mol_type = other DNA
tcttatgcttctatattccgtgccgtcggttccctccctc

SEQ ID NO: 46 - DNA, 45 bp, synthetic construct
  misc_feature 1..45: note = Synthetic Polynucleotide
  source 1..45: mol_type = other DNA
tgcttctatattccgaacacgttattgccgtcggttccctccctc

SEQ ID NO: 47 - DNA, 65 bp, synthetic construct
  misc_feature 1..65: note = Synthetic Polynucleotide
  source 1..65: mol_type = other DNA
tgcttctatattccgaggttcgaaggttacgtaccaacacgttattgccgtcggttccctccctc

SEQ ID NO: 48 - DNA, 65 bp, synthetic construct
  misc_feature 1..65: note = Synthetic Polynucleotide
  source 1..65: mol_type = other DNA
tgcttctatattccgcccccccccccccccccccccccccccccccccccccccctccctccctc

SEQ ID NO: 49 - DNA, 35 bp, synthetic construct
  misc_feature 1..35: note = Synthetic Polynucleotide
  source 1..35: mol_type = other DNA
tgcttctatattccgcccccccccctccctccctc

SEQ ID NO: 50 - DNA, 55 bp, synthetic construct
  misc_feature 1..55: note = Synthetic Polynucleotide
  source 1..55: mol_type = other DNA
tgcttctatattccggttacgtaccaacacgttattgccgtcggttccctccctc

SEQ ID NO: 51 - DNA, 35 bp, synthetic construct
  misc_feature 1..35: note = Synthetic Polynucleotide
  source 1..35: mol_type = other DNA
tgcttctatattccgtgccgtcggttccctccctc

SEQ ID NO: 52 - DNA, 40 bp, synthetic construct
  misc_feature 1..40: note = Synthetic Polynucleotide
  source 1..40: mol_type = other DNA
tttttttcccaacacgttattgccgtcggttccctccctc

SEQ ID NO: 53 - DNA, 60 bp, synthetic construct
  misc_feature 1..60: note = Synthetic Polynucleotide
  source 1..60: mol_type = other DNA
ttttttttttaggttcgaaggttacgtaccaacacgttattgccgtcggttccctccctc

SEQ ID NO: 54 - DNA, 60 bp, synthetic construct
  misc_feature 1..60: note = Synthetic Polynucleotide
  source 1..60: mol_type = other DNA
ttttttttttcccccccccccccccccccccccccccccccccccccccctccctccctc

SEQ ID NO: 55 - DNA, 30 bp, synthetic construct
  misc_feature 1..30: note = Synthetic Polynucleotide
  source 1..30: mol_type = other DNA
ttttttttttcccccccccctccctccctc

SEQ ID NO: 56 - DNA, 50 bp, synthetic construct
  misc_feature 1..50: note = Synthetic Polynucleotide
  source 1..50: mol_type = other DNA
ttttttttttgttacgtaccaacacgttattgccgtcggttccctccctc

SEQ ID NO: 57 - DNA, 30 bp, synthetic construct
  misc_feature 1..30: note = Synthetic Polynucleotide
  source 1..30: mol_type = other DNA
tttttttttttgccgtcggttccctccctc

SEQ ID NO: 58 - DNA, 45 bp, synthetic construct
  misc_feature 1..45: note = Synthetic Polynucleotide
  source 1..45: mol_type = other DNA
ttttttttttttcccaacacgttattgccgtcggttccctccctc

SEQ ID NO: 59 - DNA, 65 bp, synthetic construct
  misc_feature 1..65: note = Synthetic Polynucleotide
  source 1..65: mol_type = other DNA
tttttttttttttttaggttcgaaggttacgtaccaacacgttattgccgtcggttccctccctc

SEQ ID NO: 60 - DNA, 65 bp, synthetic construct
  misc_feature 1..65: note = Synthetic Polynucleotide
  source 1..65: mol_type = other DNA
tttttttttttttttcccccccccccccccccccccccccccccccccccccccctccctccctc

SEQ ID NO: 61 - DNA, 35 bp, synthetic construct
  misc_feature 1..35: note = Synthetic Polynucleotide
  source 1..35: mol_type = other DNA
tttttttttttttttcccccccccctccctccctc

SEQ ID NO: 62 - DNA, 55 bp, synthetic construct
  misc_feature 1..55: note = Synthetic Polynucleotide
  source 1..55: mol_type = other DNA
tttttttttttttttgttacgtaccaacacgttattgccgtcggttccctccctc

SEQ ID NO: 63 - DNA, 35 bp, synthetic construct
  misc_feature 1..35: note = Synthetic Polynucleotide
  source 1..35: mol_type = other DNA
ttttttttttttttttgccgtcggttccctccctc

SEQ ID NO: 64 - DNA, 50 bp, synthetic construct
  misc_feature 1..50: note = Synthetic Polynucleotide
  source 1..50: mol_type = other DNA
tttttttttttttttttcccaacacgttattgccgtcggttccctccctc

SEQ ID NO: 65 - DNA, 70 bp, synthetic construct
  misc_feature 1..70: note = Synthetic Polynucleotide
  source 1..70: mol_type = other DNA
ttttttttttttttttttttaggttcgaaggttacgtaccaacacgttattgccgtcggttccctccctc

SEQ ID NO: 66 - DNA, 70 bp, synthetic construct
  misc_feature 1..70: note = Synthetic Polynucleotide
  source 1..70: mol_type = other DNA
ttttttttttttttttttttcccccccccccccccccccccccccccccccccccccccctccctccctc

SEQ ID NO: 67 - DNA, 40 bp, synthetic construct
  misc_feature 1..40: note = Synthetic Polynucleotide
  source 1..40: mol_type = other DNA
ttttttttttttttttttttcccccccccctccctccctc

SEQ ID NO: 68 - DNA, 60 bp, synthetic construct
  misc_feature 1..60: note = Synthetic Polynucleotide
  source 1..60: mol_type = other DNA
ttttttttttttttttttttgttacgtaccaacacgttattgccgtcggttccctccctc

SEQ ID NO: 69 - DNA, 40 bp, synthetic construct
  misc_feature 1..40: note = Synthetic Polynucleotide
  source 1..40: mol_type = other DNA
tttttttttttttttttttttgccgtcggttccctccctc